European Patent Application EP 4 553 160 A1, published May 14, 2025. Title: ANTIVIRAL AGENTS, PHARMACEUTICAL COMPOSITIONS FOR TREATING OR PREVENTING VIRAL INFECTIONS, KITS FOR ASSESSING THE RISK OF SEVERE VIRAL INFECTIONS, AND METHODS FOR ASSESSING THE RISK OF SEVERE VIRAL INFECTIONS. Applicant: 国立大学法人東北大学. The sequence listing filed with the application follows.

SEQUENCE LISTING (22 sequences)

SEQ ID NO: 1 - DNA, 1524 bp, Homo sapiens
  source 1..1524: mol_type = genomic DNA
atgctgcgccgcgctctgctgtgcctggccgtggccgccctggtgcgcgccgacgcccccgaggaggaggaccacgtcctggtgctgcggaaaagcaacttcgcggaggcgctggcggcccacaagtacctgctggtggagttctatgccccttggtgtggccactgcaaggctctggcccctgagtatgccaaagccgctgggaagctgaaggcagaaggttccgagatcaggttggccaaggtggacgccacggaggagtctgacctggcccagcagtacggcgtgcgcggctatcccaccatcaagttcttcaggaatggagacacggcttcccccaaggaatatacagctggcagagaggctgatgacatcgtgaactggctgaagaagcgcacgggcccggctgccaccaccctgcctgacggcgcagctgcagagtccttggtggagtccagcgaggtggctgtcatcggcttcttcaaggacgtggagtcggactctgccaagcagtttttgcaggcagcagaggccatcgatgacataccatttgggatcacttccaacagtgacgtgttctccaaataccagctcgacaaagatggggttgtcctctttaagaagtttgatgaaggccggaacaactttgaaggggaggtcaccaaggagaacctgctggactttatcaaacacaaccagctgccccttgtcatcgagttcaccgagcagacagccccgaagatttttggaggtgaaatcaagactcacatcctgctgttcttgcccaagagtgtgtctgactatgacggcaaactgagcaacttcaaaacagcagccgagagcttcaagggcaagatcctgttcatcttcatcgacagcgaccacaccgacaaccagcgcatcctcgagttctttggcctgaagaaggaagagtgcccggccgtgcgcctcatcaccctggaggaggagatgaccaagtacaagcccgaatcggaggagctgacggcagagaggatcacagagttctgccaccgcttcctggagggcaaaatcaagccccacctgatgagccaggagctgccggaggactgggacaagcagcctgtcaaggtgcttgttgggaagaactttgaagacgtggcttttgatgagaaaaaaaacgtctttgtggagttctatgccccatggtgtggtcactgcaaacagttggctcccatttgggataaactgggagagacgtacaaggaccatgagaacatcgtcatcgccaagatggactcgactgccaacgaggtggaggccgtcaaagtgcacagcttccccacactcaagttctttcctgccagtgccgacaggacggtcattgattacaacggggaacgcacgctggatggttttaagaaattcctggagagcggtggccaggatggggcaggggatgatgacgatctcgaggacctggaagaagcagaggagccagacatggaggaagacgatgatcagaaagctgtgaaagatgaactg

SEQ ID NO: 2 - protein, 508 aa, Homo sapiens
MLRRALLCLAVAALVRADAPEEEDHVLVLRKSNFAEALAAHKYLLVEFYAPWCGHCKALAPEYAKAAGKLKAEGSEIRLAKVDATEESDLAQQYGVRGYPTIKFFRNGDTASPKEYTAGREADDIVNWLKKRTGPAATTLPDGAAAESLVESSEVAVIGFFKDVESDSAKQFLQAAEAIDDIPFGITSNSDVFSKYQLDKDGVVLFKKFDEGRNNFEGEVTKENLLDFIKHNQLPLVIEFTEQTAPKIFGGEIKTHILLFLPKSVSDYDGKLSNFKTAAESFKGKILFIFIDSDHTDNQRILEFFGLKKEECPAVRLITLEEEMTKYKPESEELTAERITEFCHRFLEGKIKPHLMSQELPEDWDKQPVKVLVGKNFEDVAFDEKKNVFVEFYAPWCGHCKQLAPIWDKLGETYKDHENIVIAKMDSTANEVEAVKVHSFPTLKFFPASADRTVIDYNGERTLDGFKKFLESGGQDGAGDDDDLEDLEEAEEPDMEEDDDQKAVKDEL

SEQ ID NO: 3 - DNA, 1536 bp, Homo sapiens
  source 1..1536: mol_type = genomic DNA
atgggcagcagccatcatcatcatcatcacagcagcggcctggtgccgcgcggcagccatatggacgcccccgaggaggaggaccacgtcctggtgctgcggaaaagcaacttcgcggaggcgctggcggcccacaagtacctgctggtggagttctatgccccttggtgtggccactgcaaggctctggcccctgagtatgccaaagccgctgggaagctgaaggcagaaggttccgagatcaggttggccaaggtggacgccacggaggagtctgacctggcccagcagtacggcgtgcgcggctatcccaccatcaagttcttcaggaatggagacacggcttcccccaaggaatatacagctggcagagaggctgatgacatcgtgaactggctgaagaagcgcacgggcccggctgccaccaccctgcctgacggcgcagctgcagagtccttggtggagtccagcgaggtggctgtcatcggcttcttcaaggacgtggagtcggactctgccaagcagtttttgcaggcagcagaggccatcgatgacataccatttgggatcacttccaacagtgacgtgttctccaaataccagctcgacaaagatggggttgtcctctttaagaagtttgatgaaggccggaacaactttgaaggggaggtcaccaaggagaacctgctggactttatcaaacacaaccagctgccccttgtcatcgagttcaccgagcagacagccccgaagatttttggaggtgaaatcaagactcacatcctgctgttcttgcccaagagtgtgtctgactatgacggcaaactgagcaacttcaaaacagcagccgagagcttcaagggcaagatcctgttcatcttcatcgacagcgaccacaccgacaaccagcgcatcctcgagttctttggcctgaagaaggaagagtgcccggccgtgcgcctcatcaccctggaggaggagatgaccaagtacaagcccgaatcggaggagctgacggcagagaggatcacagagttctgccaccgcttcctggagggcaaaatcaagccccacctgatgagccaggagctgccggaggactgggacaagcagcctgtcaaggtgcttgttgggaagaactttgaagacgtggcttttgatgagaaaaaaaacgtctttgtggagttctatgccccatggtgtggtcactgcaaacagttggctcccatttgggataaactgggagagacgtacaaggaccatgagaacatcgtcatcgccaagatggactcgactgccaacgaggtggaggccgtcaaagtgcacagcttccccacactcaagttctttcctgccagtgccgacaggacggtcattgattacaacggggaacgcacgctggatggttttaagaaattcctggagagcggtggccaggatggggcaggggatgatgacgatctcgaggacctggaagaagcagaggagccagacatggaggaagacgatgatcagaaagctgtgaaagatgaactg

SEQ ID NO: 4 - protein, 512 aa, Homo sapiens
MGSSHHHHHHSSGLVPRGSHMDAPEEEDHVLVLRKSNFAEALAAHKYLLVEFYAPWCGHCKALAPEYAKAAGKLKAEGSEIRLAKVDATEESDLAQQYGVRGYPTIKFFRNGDTASPKEYTAGREADDIVNWLKKRTGPAATTLPDGAAAESLVESSEVAVIGFFKDVESDSAKQFLQAAEAIDDIPFGITSNSDVFSKYQLDKDGVVLFKKFDEGRNNFEGEVTKENLLDFIKHNQLPLVIEFTEQTAPKIFGGEIKTHILLFLPKSVSDYDGKLSNFKTAAESFKGKILFIFIDSDHTDNQRILEFFGLKKEECPAVRLITLEEEMTKYKPESEELTAERITEFCHRFLEGKIKPHLMSQELPEDWDKQPVKVLVGKNFEDVAFDEKKNVFVEFYAPWCGHCKQLAPIWDKLGETYKDHENIVIAKMDSTANEVEAVKVHSFPTLKFFPASADRTVIDYNGERTLDGFKKFLESGGQDGAGDDDDLEDLEEAEEPDMEEDDDQKAVKDEL

SEQ ID NO: 5 - DNA, 1296 bp, Homo sapiens
  source 1..1296: mol_type = genomic DNA
atgcccgcgcgcccaggacgcctcctcccgctgctggcccggccggcggccctgactgcgctgctgctgctgctgctgggccatggcggcggcgggcgctggggcgcccgggcccaggaggcggcggcggcggcggcggacgggccccccgcggcagacggcgaggacggacaggacccgcacagcaagcacctgtacacggccgacatgttcacgcacgggatccagagcgccgcgcacttcgtcatgttcttcgcgccctggtgtggacactgccagcggctgcagccgacttggaatgacctgggagacaaatacaacagcatggaagatgccaaagtctatgtggctaaagtggactgcacggcccactccgacgtgtgctccgcccagggggtgcgaggataccccaccttaaagcttttcaagccaggccaagaagctgtgaagtaccagggtcctcgggacttccagacactggaaaactggatgctgcagacactgaacgaggagccagtgacaccagagccggaagtggaaccgcccagtgcccccgagctcaagcaagggctgtatgagctctcagcaagcaactttgagctgcacgttgcacaaggcgaccactttatcaagttcttcgctccgtggtgtggtcactgcaaagccctggctccaacctgggagcagctggctctgggccttgaacattccgaaactgtcaagattggcaaggttgattgtacacagcactatgaactctgctccggaaaccaggttcgtggctatcccactcttctctggttccgagatgggaaaaaggtggatcagtacaagggaaagcgggatttggagtcactgagggagtacgtggagtcgcagctgcagcgcacagagactggagcgacggagaccgtcacgccctcagaggccccggtgctggcagctgagcccgaggctgacaagggcactgtgttggcactcactgaaaataacttcgatgacaccattgcagaaggaataaccttcatcaagttttatgctccatggtgtggtcattgtaagactctggctcctacttgggaggaactctctaaaaaggaattccctggtctggcgggggtcaagatcgccgaagtagactgcactgctgaacggaatatctgcagcaagtattcggtacgaggctaccccacgttattgcttttccgaggagggaagaaagtcagtgagcacagtggaggcagagaccttgactcgttacaccgctttgtcctgagccaagcgaaagacgaactt

SEQ ID NO: 6 - protein, 432 aa, Homo sapiens
MPARPGRLLPLLARPAALTALLLLLLGHGGGGRWGARAQEAAAAAADGPPAADGEDGQDPHSKHLYTADMFTHGIQSAAHFVMFFAPWCGHCQRLQPTWNDLGDKYNSMEDAKVYVAKVDCTAHSDVCSAQGVRGYPTLKLFKPGQEAVKYQGPRDFQTLENWMLQTLNEEPVTPEPEVEPPSAPELKQGLYELSASNFELHVAQGDHFIKFFAPWCGHCKALAPTWEQLALGLEHSETVKIGKVDCTQHYELCSGNQVRGYPTLLWFRDGKKVDQYKGKRDLESLREYVESQLQRTETGATETVTPSEAPVLAAEPEADKGTVLALTENNFDDTIAEGITFIKFYAPWCGHCKTLAPTWEELSKKEFPGLAGVKIAEVDCTAERNICSKYSVRGYPTLLLFRGGKKVSEHSGGRDLDSLHRFVLSQAKDEL

SEQ ID NO: 7 - DNA, 1263 bp, Homo sapiens
  source 1..1263: mol_type = genomic DNA
atgggcagcagccatcatcatcatcatcacagcagcggcctggtgccgcgcggcagccatatgcgctggggcgcccgggcccaggaggcggcggcggcggcggcggacgggccccccgcggcagacggcgaggacggacaggacccgcacagcaagcacctgtacacggccgacatgttcacgcacggaatccagagcgccgcgcacttcgtcatgttcttcgcgccctggtgtggacactgccagcggctgcagccgacttggaatgacctgggagacaaatacaacagcatggaagatgccaaagtctatgtggctaaagtggactgcacggcccactccgacgtgtgctccgcccagggggtgcgaggataccccaccttaaagcttttcaagccaggccaagaagctgtgaagtaccagggtcctcgggacttccagacactggaaaactggatgctgcagacactgaacgaggagccagtgacaccagagccggaagtggaaccgcccagtgcccccgagctcaagcaagggctgtatgagctctcagcaagcaactttgagctgcacgttgcacaaggcgaccactttatcaagttcttcgctccgtggtgtggtcactgcaaagccctggctccaacctgggagcagctggctctgggccttgaacattccgaaactgtcaagattggcaaggttgattgtacacagcactatgaactctgctccggaaaccaggttcgtggctatcccactcttctctggttccgagatgggaaaaaggtggatcagtacaagggaaagcgggatttggagtcactgagggagtacgtggagtcgcagctgcagcgcacagagactggagcgacggagaccgtcacgccctcagaggccccggtgctggcagctgagcccgaggctgacaagggcactgtgttggcactcactgaaaataacttcgatgacaccattgcagaaggaataaccttcatcaagttttatgctccatggtgtggtcattgtaagactctggctcctacttgggaggaactctctaaaaaggaattccctggtctggcgggggtcaagatcgccgaagtagactgcactgctgaacggaatatctgcagcaagtattcggtacgaggctaccccacgttattgcttttccgaggagggaagaaagtcagtgagcacagtggaggcagagaccttgactcgttacaccgctttgtcctgagccaagcgaaagacgaactt

SEQ ID NO: 8 - protein, 421 aa, Homo sapiens
MGSSHHHHHHSSGLVPRGSHMRWGARAQEAAAAAADGPPAADGEDGQDPHSKHLYTADMFTHGIQSAAHFVMFFAPWCGHCQRLQPTWNDLGDKYNSMEDAKVYVAKVDCTAHSDVCSAQGVRGYPTLKLFKPGQEAVKYQGPRDFQTLENWMLQTLNEEPVTPEPEVEPPSAPELKQGLYELSASNFELHVAQGDHFIKFFAPWCGHCKALAPTWEQLALGLEHSETVKIGKVDCTQHYELCSGNQVRGYPTLLWFRDGKKVDQYKGKRDLESLREYVESQLQRTETGATETVTPSEAPVLAAEPEADKGTVLALTENNFDDTIAEGITFIKFYAPWCGHCKTLAPTWEELSKKEFPGLAGVKIAEVDCTAERNICSKYSVRGYPTLLLFRGGKKVSEHSGGRDLDSLHRFVLSQAKDEL

SEQ ID NO: 9 - DNA, 1515 bp, Homo sapiens
  source 1..1515: mol_type = genomic DNA
atgcgcctccgccgcctagcgctgttcccgggtgtggcgctgcttcttgccgcggcccgcctcgccgctgcctccgacgtgctagaactcacggacgacaacttcgagagtcgcatctccgacacgggctctgcgggcctcatgctcgtcgagttcttcgccccctggtgtggacactgcaagagacttgcacctgagtatgaagctgcagctaccagattaaaaggaatagtcccattagcaaaggttgattgcactgccaacactaacacctgtaataaatatggagtcagtggatatccaaccctgaagatatttagagatggtgaagaagcaggtgcttatgatggacctaggactgctgatggaattgtcagccacttgaagaagcaggcaggaccagcttcagtgcctctcaggactgaggaagaatttaagaaattcattagtgataaagatgcctctatagtaggttttttcgatgattcattcagtgaggctcactccgagttcctaaaagcagccagcaacttgagggataactaccgatttgcacatacgaatgttgagtctctggtgaacgagtatgatgataatggagagggtatcatcttatttcgtccttcacatctcactaacaagtttgaggacaagactgtggcatatacagagcaaaaaatgaccagtggcaaaattaaaaagtttatccaggaaaacatttttggtatctgccctcacatgacagaagacaataaagatttgatacagggcaaggacttacttattgcttactatgatgtggactatgaaaagaacgctaaaggttccaactactggagaaacagggtaatgatggtggcaaagaaattcctggatgctgggcacaaactcaactttgctgtagctagccgcaaaacctttagccatgaactttctgattttggcttggagagcactgctggagagattcctgttgttgctatcagaactgctaaaggagagaagtttgtcatgcaggaggagttctcgcgtgatgggaaggctctggagaggttcctgcaggattactttgatggcaatctgaagagatacctgaagtctgaacctatcccagagagcaatgatgggcctgtgaaggtagtggtagcagagaattttgatgaaatagtgaataatgaaaataaagatgtgctgattgaattttatgccccttggtgtggtcactgtaagaacctggagcccaagtataaagaacttggcgagaagctcagcaaagacccaaatatcgtcatagccaagatggatgccacagccaatgatgtgccttctccatatgaagtcagaggttttcctaccatatacttctctccagccaacaagaagctaaatccaaagaaatatgaaggtggccgtgaattaagtgattttattagctatctacaaagagaagctacaaacccccctgtaattcaagaagaaaaacccaagaagaagaagaaggcacaggaggatctc

SEQ ID NO: 10 - protein, 505 aa, Homo sapiens
MRLRRLALFPGVALLLAAARLAAASDVLELTDDNFESRISDTGSAGLMLVEFFAPWCGHCKRLAPEYEAAATRLKGIVPLAKVDCTANTNTCNKYGVSGYPTLKIFRDGEEAGAYDGPRTADGIVSHLKKQAGPASVPLRTEEEFKKFISDKDASIVGFFDDSFSEAHSEFLKAASNLRDNYRFAHTNVESLVNEYDDNGEGIILFRPSHLTNKFEDKTVAYTEQKMTSGKIKKFIQENIFGICPHMTEDNKDLIQGKDLLIAYYDVDYEKNAKGSNYWRNRVMMVAKKFLDAGHKLNFAVASRKTFSHELSDFGLESTAGEIPVVAIRTAKGEKFVMQEEFSRDGKALERFLQDYFDGNLKRYLKSEPIPESNDGPVKVVVAENFDEIVNNENKDVLIEFYAPWCGHCKNLEPKYKELGEKLSKDPNIVIAKMDATANDVPSPYEVRGFPTIYFSPANKKLNPKKYEGGRELSDFISYLQREATNPPVIQEEKPKKKKKAQEDL

SEQ ID NO: 11 - DNA, 1512 bp, Homo sapiens
  source 1..1512: mol_type = genomic DNA
atgggcagcagccatcatcatcatcatcacagcagcggcctggtgccgcgcggcagccatatgctcgagtccgacgtgctagaactcacggacgacaacttcgagagtcgcatctccgacacgggctctgcgggcctcatgctcgtcgagttcttcgccccctggtgtggacactgcaagagacttgcacctgagtatgaagctgcagctaccagattaaaaggaatagtcccattagcaaaggttgattgcactgccaacactaacacctgtaataaatatggagtcagtggatatccaaccctgaagatatttagagatggtgaagaagcaggtgcttatgatggacctaggactgctgatggaattgtcagccacttgaagaagcaggcaggaccagcttcagtgcctctcaggactgaggaagaatttaagaaattcattagtgataaagatgcctctatagtaggttttttcgatgattcattcagtgaggctcactccgagttcctaaaagcagccagcaacttgagggataactaccgatttgcacatacgaatgttgagtctctggtgaacgagtatgatgataatggagagggtatcatcttatttcgtccttcacatctcactaacaagtttgaggacaagactgtggcatatacagagcaaaaaatgaccagtggcaaaattaaaaagtttatccaggaaaacatttttggtatctgccctcacatgacagaagacaataaagatttgatacagggcaaggacttacttattgcttactatgatgtggactatgaaaagaacgctaaaggttccaactactggagaaacagggtaatgatggtggcaaagaaattcctggatgctgggcacaaactcaactttgctgtagctagccgcaaaacctttagccatgaactttctgattttggcttggagagcactgctggagagattcctgttgttgctatcagaactgctaaaggagagaagtttgtcatgcaggaggagttctcgcgtgatgggaaggctctggagaggttcctgcaggattactttgatggcaatctgaagagatacctgaagtctgaacctatcccagagagcaatgatgggcctgtgaaggtagtggtagcagagaattttgatgaaatagtgaataatgaaaataaagatgtgctgattgaattttatgccccttggtgtggtcactgtaagaacctggagcccaagtataaagaacttggcgagaagctcagcaaagacccaaatatcgtcatagccaagatggatgccacagccaatgatgtgccttctccatatgaagtcagaggttttcctaccatatacttctctccagccaacaagaagctaaatccaaagaaatatgaaggtggccgtgaattaagtgattttattagctatctacaaagagaagctacaaacccccctgtaattcaagaagaaaaacccaagaagaagaagaaggcacaggaggatctc

SEQ ID NO: 12 - protein, 504 aa, Homo sapiens
MGSSHHHHHHSSGLVPRGSHMLESDVLELTDDNFESRISDTGSAGLMLVEFFAPWCGHCKRLAPEYEAAATRLKGIVPLAKVDCTANTNTCNKYGVSGYPTLKIFRDGEEAGAYDGPRTADGIVSHLKKQAGPASVPLRTEEEFKKFISDKDASIVGFFDDSFSEAHSEFLKAASNLRDNYRFAHTNVESLVNEYDDNGEGIILFRPSHLTNKFEDKTVAYTEQKMTSGKIKKFIQENIFGICPHMTEDNKDLIQGKDLLIAYYDVDYEKNAKGSNYWRNRVMMVAKKFLDAGHKLNFAVASRKTFSHELSDFGLESTAGEIPVVAIRTAKGEKFVMQEEFSRDGKALERFLQDYFDGNLKRYLKSEPIPESNDGPVKVVVAENFDEIVNNENKDVLIEFYAPWCGHCKNLEPKYKELGEKLSKDPNIVIAKMDATANDVPSPYEVRGFPTIYFSPANKKLNPKKYEGGRELSDFISYLQREATNPPVIQEEKPKKKKKAQEDL

SEQ ID NO: 13 - DNA, 1935 bp, Homo sapiens
  source 1..1935: mol_type = genomic DNA
atgaggccccggaaagccttcctgctcctgctgctcttggggctggtgcagctgctggccgtggcgggtgccgagggcccggacgaggattcttctaacagagaaaatgccattgaggatgaagaggaggaggaggaggaagatgatgatgaggaagaagacgacttggaagttaaggaagaaaatggagtcttggtcctaaatgatgcaaactttgataattttgtggctgacaaagacacagtgctgctggagttttatgctccatggtgtggacattgcaagcagtttgctccggaatatgaaaaaattgccaacatattaaaggataaagatcctcccattcctgttgccaagatcgatgcaacctcagcgtctgtgctggccagcaggtttgatgtgagtggctaccccaccatcaagatccttaagaaggggcaggctgtagactacgagggctccagaacccaggaagaaattgttgccaaggtcagagaagtctcccagcccgactggacgcctccaccagaagtcacgcttgtgttgaccaaagagaactttgatgaagttgtgaatgatgcagatatcattctggtggagttttatgccccatggtgtggacactgcaagaaacttgcccccgagtatgagaaggccgccaaggagctcagcaagcgttctcctccaattcccctggcaaaggtcgacgccaccgcagaaacagacctggccaagaggtttgatgtctctggctatcccaccctgaaaattttccgcaaaggaaggccttatgactacaacggcccacgagaaaaatatggaatcgttgattacatgatcgagcagtccgggcctccctccaaggagattctgaccctgaagcaggtccaggagttcctgaaggatggagacgatgtcatcatcatcggggtctttaagggggagagtgacccagcctaccagcaataccaggatgccgctaacaacctgagagaagattacaaatttcaccacactttcagcacagaaatagcaaagttcttgaaagtctcccaggggcagttggttgtaatgcagcctgagaaattccagtccaagtatgagccccggagccacatgatggacgtccagggctccacccaggactcggccatcaaggacttcgtgctgaagtacgccctgcccctggttggccaccgcaaggtgtcaaacgatgctaagcgctacaccaggcgccccctggtggtcgtctactacagtgtggacttcagctttgattacagagctgcaactcagttttggcggagcaaagtcctagaggtggccaaggacttccctgagtacacctttgccattgcggacgaagaggactatgctggggaggtgaaggacctggggctcagcgagagtggggaggatgtcaatgccgccatcctggacgagagtgggaagaagttcgccatggagccagaggagtttgactctgacaccctccgcgagtttgtcactgctttcaaaaaaggaaaactgaagccagtcatcaaatcccagccagtgcccaagaacaacaagggacccgtcaaggtcgtggtgggaaagacctttgactccattgtgatggaccccaagaaggacgtcctcatcgagttctacgcgccatggtgcgggcactgcaagcagctagagcccgtgtacaacagcctggccaagaagtacaagggccaaaagggcctggtcatcgccaagatggacgccactgccaacgacgtccccagcgaccgctataaggtggagggcttccccaccatctacttcgcccccagtggggacaaaaagaacccagttaaatttgagggtggagacagagatctggagcatttgagcaagtttatagaagaacatgccacaaaactgagcaggaccaaggaagagctt

SEQ ID NO: 14 - protein, 645 aa, Homo sapiens
MRPRKAFLLLLLLGLVQLLAVAGAEGPDEDSSNRENAIEDEEEEEEEDDDEEEDDLEVKEENGVLVLNDANFDNFVADKDTVLLEFYAPWCGHCKQFAPEYEKIANILKDKDPPIPVAKIDATSASVLASRFDVSGYPTIKILKKGQAVDYEGSRTQEEIVAKVREVSQPDWTPPPEVTLVLTKENFDEVVNDADIILVEFYAPWCGHCKKLAPEYEKAAKELSKRSPPIPLAKVDATAETDLAKRFDVSGYPTLKIFRKGRPYDYNGPREKYGIVDYMIEQSGPPSKEILTLKQVQEFLKDGDDVIIIGVFKGESDPAYQQYQDAANNLREDYKFHHTFSTEIAKFLKVSQGQLVVMQPEKFQSKYEPRSHMMDVQGSTQDSAIKDFVLKYALPLVGHRKVSNDAKRYTRRPLVVVYYSVDFSFDYRAATQFWRSKVLEVAKDFPEYTFAIADEEDYAGEVKDLGLSESGEDVNAAILDESGKKFAMEPEEFDSDTLREFVTAFKKGKLKPVIKSQPVPKNNKGPVKVVVGKTFDSIVMDPKKDVLIEFYAPWCGHCKQLEPVYNSLAKKYKGQKGLVIAKMDATANDVPSDRYKVEGFPTIYFAPSGDKKNPVKFEGGDRDLEHLSKFIEEHATKLSRTKEEL

SEQ ID NO: 15 - DNA, 1923 bp, Homo sapiens
  source 1..1923: mol_type = genomic DNA
atgggcagcagccatcatcatcatcatcacagcagcggcctggtgccgcgcggcagccatgagggcccggacgaggattcttctaacagagaaaatgccattgaggatgaagaggaggaggaggaggaagatgatgatgaggaagaagacgacttggaagttaaggaagaaaatggagtcttggtcctaaatgatgcaaactttgataattttgtggctgacaaagacacagtgctgctggagttttatgctccatggtgtggacattgcaagcagtttgctccggaatatgaaaaaattgccaacatattaaaggataaagatcctcccattcctgttgccaagatcgatgcaacctcagcgtctgtgctggccagcaggtttgatgtgagtggctaccccaccatcaagatccttaagaaggggcaggctgtagactacgagggctccagaacccaggaagaaattgttgccaaggtcagagaagtctcccagcccgactggacgcctccaccagaagtcacgcttgtgttgaccaaagagaactttgatgaagttgtgaatgatgcagatatcattctggtggagttttatgccccatggtgtggacactgcaagaaacttgcccccgagtatgagaaggccgccaaggagctcagcaagcgttctcctccaattcccctggcaaaggtcgacgccaccgcagaaacagacctggccaagaggtttgatgtctctggctatcccaccctgaaaattttccgcaaaggaaggccttatgactacaacggcccacgagaaaaatatggaatcgttgattacatgatcgagcagtccgggcctccctccaaggagattctgaccctgaagcaggtccaggagttcctgaaggatggagacgatgtcatcatcatcggggtctttaagggggagagtgacccagcctaccagcaataccaggatgccgctaacaacctgagagaagattacaaatttcaccacactttcagcacagaaatagcaaagttcttgaaagtctcccaggggcagttggttgtaatgcagcctgagaaattccagtccaagtatgagccccggagccacatgatggacgtccagggctccacccaggactcggccatcaaggacttcgtgctgaagtacgccctgcccctggttggccaccgcaaggtgtcaaacgatgctaagcgctacaccaggcgccccctggtggtcgtctactacagtgtggacttcagctttgattacagagctgcaactcagttttggcggagcaaagtcctagaggtggccaaggacttccctgagtacacctttgccattgcggacgaagaggactatgctggggaggtgaaggacctggggctcagcgagagtggggaggatgtcaatgccgccatcctggacgagagtgggaagaagttcgccatggagccagaggagtttgactctgacaccctccgcgagtttgtcactgctttcaaaaaaggaaaactgaagccagtcatcaaatcccagccagtgcccaagaacaacaagggacccgtcaaggtcgtggtgggaaagacctttgactccattgtgatggaccccaagaaggacgtcctcatcgagttctacgcgccatggtgcgggcactgcaagcagctagagcccgtgtacaacagcctggccaagaagtacaagggccaaaagggcctggtcatcgccaagatggacgccactgccaacgacgtccccagcgaccgctataaggtggagggcttccccaccatctacttcgcccccagtggggacaaaaagaacccagttaaatttgagggtggagacagagatctggagcatttgagcaagtttatagaagaacatgccacaaaactgagcaggaccaaggaagagctt

SEQ ID NO: 16 - protein, 641 aa, Homo sapiens
MGSSHHHHHHSSGLVPRGSHEGPDEDSSNRENAIEDEEEEEEEDDDEEEDDLEVKEENGVLVLNDANFDNFVADKDTVLLEFYAPWCGHCKQFAPEYEKIANILKDKDPPIPVAKIDATSASVLASRFDVSGYPTIKILKKGQAVDYEGSRTQEEIVAKVREVSQPDWTPPPEVTLVLTKENFDEVVNDADIILVEFYAPWCGHCKKLAPEYEKAAKELSKRSPPIPLAKVDATAETDLAKRFDVSGYPTLKIFRKGRPYDYNGPREKYGIVDYMIEQSGPPSKEILTLKQVQEFLKDGDDVIIIGVFKGESDPAYQQYQDAANNLREDYKFHHTFSTEIAKFLKVSQGQLVVMQPEKFQSKYEPRSHMMDVQGSTQDSAIKDFVLKYALPLVGHRKVSNDAKRYTRRPLVVVYYSVDFSFDYRAATQFWRSKVLEVAKDFPEYTFAIADEEDYAGEVKDLGLSESGEDVNAAILDESGKKFAMEPEEFDSDTLREFVTAFKKGKLKPVIKSQPVPKNNKGPVKVVVGKTFDSIVMDPKKDVLIEFYAPWCGHCKQLEPVYNSLAKKYKGQKGLVIAKMDATANDVPSDRYKVEGFPTIYFAPSGDKKNPVKFEGGDRDLEHLSKFIEEHATKLSRTKEEL

SEQ ID NO: 17 - DNA, 1320 bp, Homo sapiens
  source 1..1320: mol_type = genomic DNA
atggctctcctggtgctcggtctggtgagctgtaccttctttctggcagtgaatggtctgtattcctctagtgatgatgtgatcgaattaactccatcgaatttcaaccgagaagttattcagagtgatagtttgtggcttgtagaattctatgctccatggtgtggtcactgtcaaagattaacaccagaatggaagaaagcagcaactgcattaaaagatgttgtcaaagttggtgcagttgatgcagataagcatcattccctaggaggtcagtatggtgttcagggatttcctaccattaagatttttggatccaacaaaaacagaccagaagattaccaaggtggcagaactggtgaagccattgtagatgctgcgctgagtgctctgcgccagctcgtgaaggatcgcctcgggggacggagcggaggatacagttctggaaaacaaggcagaagtgatagttcaagtaagaaggatgtgattgagctgacagacgacagctttgataagaatgttctggacagtgaagatgtttggatggttgagttctatgctccttggtgtggacactgcaaaaacctagagccagagtgggctgccgcagcttcagaagtaaaagagcagacgaaaggaaaagtgaaactggcagctgtggatgctacagtcaatcaggttctggcctcccgatacgggattagaggatttcctacaatcaagatatttcagaaaggcgagtctcctgtggattatgacggtgggcggacaagatccgacatcgtgtcccgggcccttgatttgttttctgataacgccccacctcctgagctgcttgagattatcaacgaggacattgccaagaggacgtgtgaggagcaccagctctgtgttgtggctgtgctgccccatatccttgatactggagctgcaggcagaaattcttatctggaagttcttctgaagttggcagacaaatacaaaaagaaaatgtgggggtggctgtggacagaagctggagcccagtctgaacttgagaccgcgttggggattggagggtttgggtaccccgccatggccgccatcaatgcacgcaagatgaaatttgctctgctaaaaggctccttcagtgagcaaggcatcaacgagtttctcagggagctctcttttgggcgtggctccacggcacctgtaggaggcggggctttccctaccatcgttgagagagagccttgggacggcagggatggcgagcttcccgtggaggatgacattgacctcagtgatgtggagcttgatgacttagggaaagatgagttg

SEQ ID NO: 18 - protein, 440 aa, Homo sapiens
MALLVLGLVSCTFFLAVNGLYSSSDDVIELTPSNFNREVIQSDSLWLVEFYAPWCGHCQRLTPEWKKAATALKDVVKVGAVDADKHHSLGGQYGVQGFPTIKIFGSNKNRPEDYQGGRTGEAIVDAALSALRQLVKDRLGGRSGGYSSGKQGRSDSSSKKDVIELTDDSFDKNVLDSEDVWMVEFYAPWCGHCKNLEPEWAAAASEVKEQTKGKVKLAAVDATVNQVLASRYGIRGFPTIKIFQKGESPVDYDGGRTRSDIVSRALDLFSDNAPPPELLEIINEDIAKRTCEEHQLCVVAVLPHILDTGAAGRNSYLEVLLKLADKYKKKMWGWLWTEAGAQSELETALGIGGFGYPAMAAINARKMKFALLKGSFSEQGINEFLRELSFGRGSTAPVGGGAFPTIVEREPWDGRDGELPVEDDIDLSDVELDDLGKDEL

SEQ ID NO: 19 - DNA, 1326 bp, Homo sapiens
  source 1..1326: mol_type = genomic DNA
atgggcagcagccatcatcatcatcatcacagcagcggcctggtgccgcgcggcagccatatgctgtattcctctagtgatgatgtgatcgaattaactccatcaaatttcaaccgagaagttattcagagtgatagtttgtggcttgtagaattctatgctccatggtgtggtcactgtcaaagattaacaccagaatggaagaaagcagcaactgcattaaaagatgttgtcaaagttggtgcagttgatgcagataagcatcattccctaggaggtcagtatggtgttcagggatttcctaccattaagatttttggatccaacaaaaacagaccagaagattaccaaggtggcagaactggtgaagccattgtagatgctgcgctgagtgctctgcgccagctcgtgaaggatcgcctcgggggacggagcggaggatacagttctggaaaacaaggcagaagtgatagttcaagtaagaaggatgtgattgagctgacagacgacagctttgataagaatgttctggacagtgaagatgtttggatggttgagttctatgctccttggtgtggacactgcaaaaacctagagccagagtgggctgccgcagcttcagaagtaaaagagcagacgaaaggaaaagtgaaactggcagctgtggatgctacagtcaatcaggttctggcctcccgatacgggattagaggatttcctacaatcaagatatttcagaaaggcgagtctcctgtggattatgacggtgggcggacaagatccgacatcgtgtcccgggcccttgatttgttttctgataacgccccacctcctgagctgcttgagattatcaacgaggacattgccaagaggacgtgtgaggagcaccagctctgtgttgtggctgtgctgccccatatccttgatactggagctgcaggcagaaattcttatctggaagttcttctgaagttggcagacaaatacaaaaagaaaatgtgggggtggctgtggacagaagctggagcccagtctgaacttgagaccgcgttggggattggagggtttgggtaccccgccatggccgccatcaatgcacgcaagatgaaatttgctctgctaaaaggctccttcagtgagcaaggcatcaacgagtttctcagggagctctcttttgggcgtggctccacggcacctgtaggaggcggggctttccctaccatcgttgagagagagccttgggacggcagggatggcgagcttcccgtggaggatgacattgacctcagtgatgtggagcttgatgacttagggaaagatgagttg

SEQ ID NO: 20 - protein, 442 aa, Homo sapiens
MGSSHHHHHHSSGLVPRGSHMLYSSSDDVIELTPSNFNREVIQSDSLWLVEFYAPWCGHCQRLTPEWKKAATALKDVVKVGAVDADKHHSLGGQYGVQGFPTIKIFGSNKNRPEDYQGGRTGEAIVDAALSALRQLVKDRLGGRSGGYSSGKQGRSDSSSKKDVIELTDDSFDKNVLDSEDVWMVEFYAPWCGHCKNLEPEWAAAASEVKEQTKGKVKLAAVDATVNQVLASRYGIRGFPTIKIFQKGESPVDYDGGRTRSDIVSRALDLFSDNAPPPELLEIINEDIAKRTCEEHQLCVVAVLPHILDTGAAGRNSYLEVLLKLADKYKKKMWGWLWTEAGAQSELETALGIGGFGYPAMAAINARKMKFALLKGSFSEQGINEFLRELSFGRGSTAPVGGGAFPTIVEREPWDGRDGELPVEDDIDLSDVELDDLGKDEL

SEQ ID NO: 21 - DNA, 23 bp, synthetic construct
  source 1..23: mol_type = other DNA
agcctcttctcgttcctcatcac

SEQ ID NO: 22 - DNA, 19 bp, synthetic construct
  source 1..19: mol_type = other DNA
ccgccattgccagccattc